European Patent Specification EP 3 021 663 B1, published January 18, 2023. Title: TRANSGENIC MOUSE EXPRESSING HUMAN LIPOPROTEIN (A) WITH DISABLED VITAMIN C GENE AND ITS USE AS A DISEASE TREATMENT MODEL. Applicant: CHA , JOHN CHANG-EUN NIEDZWIECKI, ALEKSANDRA RATH, MATTHIAS  W. The sequence listing filed with the application follows.

SEQUENCE LISTING (12 sequences)

SEQ ID NO: 1 - DNA, 30 bp, Mouse
ctagtgtagtctaggtgataaggatcaact

SEQ ID NO: 2 - DNA, 25 bp, Mouse
cagctcagagagagaatgaatcaca

SEQ ID NO: 3 - DNA, 20 bp, Mouse
ctgacatcccttaggagttc

SEQ ID NO: 4 - DNA, 20 bp, Mouse
agatgtgttccaggctgcaa

SEQ ID NO: 5 - DNA, 19 bp, Mouse
cacacactgcagggtgaca

SEQ ID NO: 6 - DNA, 16 bp, Mouse
ctgcctgggtgttatc

SEQ ID NO: 7 - DNA, 25 bp, Human
cactacattttgtgccagagatgga

SEQ ID NO: 8 - DNA, 20 bp, Human
ccctgtcctgaggctcctta

SEQ ID NO: 9 - DNA, 16 bp, Human
tcagcagccctcttcc

SEQ ID NO: 10 - DNA, 24 bp, Human
aggtttaactcctcctacctccaa

SEQ ID NO: 11 - DNA, 21 bp, Human
tgagggagagggttccatctt

SEQ ID NO: 12 - DNA, 21 bp, Human
accagataacaggaagatatg